European Patent Application EP 4 417 697 A1, published August 21, 2024. Title: Modular conjugation system. Applicant: Max-Planck-Gesellschaft zur Foerderung der Wissenschaften e.V. The sequence listing filed with the application follows.

SEQUENCE LISTING (15 sequences)

SEQ ID NO: 1 - protein, 7 aa, synthetic construct
  REGION 1..7: note = linker sequence
DYDIPTT

SEQ ID NO: 2 - protein, 7 aa, synthetic construct
  REGION 1..7: note = linker sequence
GGGGGGG

SEQ ID NO: 3 - protein, 5 aa, synthetic construct
  REGION 1..5: note = linker sequence
GGGGS

SEQ ID NO: 4 - protein, 5 aa, synthetic construct
  REGION 1..5: note = linker sequence
EAAAK

SEQ ID NO: 5 - protein, 6 aa, synthetic construct
  REGION 1..6: note = His-tag His6
HHHHHH

SEQ ID NO: 6 - protein, 8 aa, synthetic construct
  REGION 1..8: note = His-tag His8
HHHHHHHH

SEQ ID NO: 7 - protein, 10 aa, synthetic construct
  REGION 1..10: note = His-tag His10
HHHHHHHHHH

SEQ ID NO: 8 - protein, 14 aa, synthetic construct
  REGION 1..14: note = His-tag His14
HHHHHHHHHHHHHH

SEQ ID NO: 9 - protein, 12 aa, synthetic construct
  REGION 1..12: note = His-tag (HisGln)6
HQHQHQHQHQHQ

SEQ ID NO: 10 - protein, 12 aa, synthetic construct
  REGION 1..12: note = His-tag (HisAsn)6
HNHNHNHNHNHN

SEQ ID NO: 11 - protein, 12 aa, synthetic construct
  REGION 1..12: note = His-tag (HisGly)5HisGln
HGHGHGHGHGHQ

SEQ ID NO: 12 - DNA, 90 bp, synthetic construct
  source 1..90: mol_type = other DNA
  misc_feature 1..90: note = CALD1_90nt_triA DNA
gtatactgctccagtctgctgtcaatcttggagactactgctgcttgatgggtcgatttgacaccactgctaaaaaagtaaacacataca

SEQ ID NO: 13 - DNA, 90 bp, synthetic construct
  source 1..90: mol_type = other DNA
  misc_feature 1..90: note = CALD1_90nt_RC_triA DNA
tgtatgtgtttacttttttagcagtggtgtcaaatcgacccatcaagcagcagtagtctccaagattgacagcagactggagcagtatac

SEQ ID NO: 14 - DNA, 60 bp, synthetic construct
  source 1..60: mol_type = other DNA
  misc_feature 1..60: note = forward primer
acactctttccctacacgacgctcttccgatctgctaatcagctagcatatgtatgagaa

SEQ ID NO: 15 - DNA, 59 bp, synthetic construct
  source 1..59: mol_type = other DNA
  misc_feature 1..59: note = reverse primer
gtgactggagttcagacgtgtgctcttccgatctttggacttgattattgtcctaagtg